European Patent Specification EP 3 596 223 B1, published June 7, 2023. Title: Branched alpha glucans. Applicant: NESTEC S.A. The sequence listing filed with the application follows.

SEQUENCE LISTING (19 sequences)

SEQ ID NO: 1 - protein, 1281 aa, Lactobacillus reuteri
  CNCM I-2452
NKGQQTTDWQKNADNQWVYNGKTDQDLKGTQYVQLPTIPDTNVQGNTNWYFVKDGIAQSGVQQWAGSYYYFDPVTYLRVDNRYVQSQWGLKYMFGKDGRIATGLYKWDKNNQWYYFNPITYLAVTNDYIQANDGNWYLFTADGTAASRVAQWAGTYYYFDPVTHLRVDNNYVQSQWGDWYLFGNDGRILSGVQQWAGTYYYFDPTTYLRVDDDYVTSQWGLKYMFGKDGRIATGLYKWDKNNQWYYFDPTTYLAVTNNYIQANDGHWYLFTADGTAASRVAKWAGTYYYFDPVTHLRVDNNYVQSQWGDWYMFGNDGRIITGRTLWYGNYYYFDPVTYLKVTNKWVDGNYYDEDGAQAISKLVTINNRLYYFDDQGKEISNQFRTIYGNTYYFGNDSAAVTGQQTIDGKVYNFSKYGHLLGNRYGKIENGKLNIYSLADNSLIKTVEAGPWENMAYSMDSNSINNIDGYISYTGWYRPYGTSQDGKTWYPTTVADWRPILMYVWPSKDVQAKFIQYFVNHGYENSNYGLTTGSVKDLSENTASIKLNEVAQNLRYVIEQHIVAAKSTSQLANDINNFITTIPELSASSELPYGQVIFVNNDNTSYADSKYRLMSRTINNQTGNDNDNSDNGYEFLTGIDIDNSNPVVQAENLNWEYFLLNYGKLMGYNPDGNFDGFRIDAADHIDADVLDQTGQLMDDMYHMKGNPQNANNHLSYNEGYRSSAARMLNKKGNPQLYMDYVGSTLGNVLGRANNRDTISNLVTGSIVNRQNDVTENEATPNWSYVTNHDSRANLINGLISKDHPGAYKAEYANQAWQEFYADQKKTDKQYAQYNVPAQYAILLSNKDTVPQIYYGDLYNETAQYMQEKSIYYDAITTLMKARKQFVSGGQTMTKLSDNLIASVRYGKGVTNANSEGTDSLSRTSGMAVIVGNNPQMAEQTISINMGRAHANEQYRNLLDTTDNGLTYNADGAENPETLTTDDNGILKVTVKGYSNPYVSGYLGVWVPVVSGNQDVTTNAATVSADSNKIFESNAALDSHMIYQDFSLYQPEPTSTENHAYNTIAQNAELFNNLGITDFWMAPPYTQYSESRYNDGYSVTDRYNLGTNANPTKYGSGEELANAIAALHSAGLKVQVDIVMNQMIGLPGQEAVTVTRADNRGIQTYVNGKTYANQMYFAYTTGGGNGQETYGGKYLSELQSKYPDLFTTRAISTGVAPDPTTRITKWSAKYENGTSLQNIGIGLAVKLPNGEYAYLRSSDNKAFNTTLPETMSSADYYANIEDD

SEQ ID NO: 2 - protein, 31 aa, Unknown
  Primer
CAGGGACCCGGTGGGCATTTACTTGGAAATC

SEQ ID NO: 3 - protein, 36 aa, Unknown
  Primer
CGAGGAGAAGCCCGGTTAATCGTCTTCAATATTAGC

SEQ ID NO: 4 - protein, 1631 aa, Streptococcus thermophilus
  NCC 2408
ICSSYFLNLPYIKKRWYNKKFIYRGEYHMEIKKRFKLYKSGKQWIRASISTVAISTGLILGGGVVHAAENQPGGTQHSVINTTNNQDQENGKQDNSLANTNENGSTKENNGQANALSQLNKVNNNATPQADNTAAVNNNATPQADNAAANDYNHSDNGNYGYIDSATINNNQLHVVGWSATNQAVNKDTSRYVIVYDDTTKSELGRVQVTNPVARPDVKKAYNVYNAQNSGFDVNVSLNFDKMNSYRDAIRIISRYSGVPDGNSDYVDYVSQPVVLDENDYAYLDNFNVNNGILHVSGWHATNKAIKRPNHFVILYDRTTNCEVARQRVITGIERPDVERAYPQVVNANISGFAADFDVTNLNPNDEYQILSRYSNRDNGEGSYVTHWFNPQRLVPTTQFNGGYLDNFNISKAGQVAVSGWHATNLSNIQSNRFVILFDNTANRQVASVKISGTDRPDVEKAYSQVLNAGKSGYNVTFDLNQSQIAQLLANHSYSIVSRYSADANGDGNNKQHTDIWSAPIVLDKTASYIDGISLNSNKLNITGWMASDASATQTNPYVIVLNDGKEVTRQKLTLTARPDVARVYPDIYNSSVSGFNTTINLTVPELNQLTGNMQVLLRYSANSDGNPTRNGDTTDQYSKSYATNGGNFDFVKVDNNQVEFSGWHASDQATDKPYQWIIVLANGKEVGRQLISSTTYGLVSYNRPDVYNVNPAISDSSTSGFHGIITLNSSIKNVPVQLVHRFSDDGQNGERNRVDFWSEVMPVASTFQKGSDQVMKNLVAKPQGNQLNIYNGNTVLKTLGPGTWENMAFAHDSSAINNIDGYLSYTGWYRPYGTSQDGKTWYQTTAMDWRPLLMYIWPSKDVQAQFIKYFVKNGYENADYGLTEASVANLNKDTDATVLNTAAQNLRYVIEQSIATNKGTRKLANDINGFVATVPELSTSSELPDESGYGQVIFVNNDNTSYADSKYRLMNRTVNNQTGNDDSDYRPEFLVGTDVDNSNPVVQAENLNWEYFLLNYGKLMGYNPDGNFDGFRIDATDHIDADVLDQMGQLMNAMYHMKGNPQNANNHLSYNEQYSRGAARMLNKKGNPQLYMDSEVFGTLENVLGRANNRYDISHLITDSIVNRQNDVTENEATPNWSFVTNHDQRNNLINGLISKDHPDMGSAYKAEYANQAWQEFYADQKKTDKQYAKYNVPAQYAILLSNKDTVPQIYYGDLYNETAQYMQEKSIYYDAITTLMKARKQFISGGQTMTKLSDNLIASVRYGKGVANANSEGTDSLSRTSGMAVIVGNNPQMAEQTISINMGRAHANEQYRNLLDTTDNGLTYNADGAKNPETLTTDDNGILKVTVKGYSNPYVSGYLGVWVPVVSGNQDVTTNAATVSADSNKIFESNAALDSHMIYQSFSLHQPKPTSTENHAYNIIAQNAELFNNLGITDFWMPPAYTSDENSRYNEGYAVTDRYNLGTNANPTKYGSGEELANAIAALHSAGLKVQADIVLNHMMGLPGQEAVTVTRASDRGMQVYVNGKTYANQIYFAYTRGGGEGQKNYGGKYLDELQKKYPELFTTKAVSTGVAPDPSVHITEWSAKYQNGTILQNIGIGLAVKLANGDYAYLRSSDNKSFNTLLPSEIAL

SEQ ID NO: 5 - protein, 1282 aa, Lactobacillus delbrueckii subsp. delbrueckii
  NCC 828
MNSRKKMMNEPSSEKQRWSLRKISVGMTSVLLGATMFWASGAGSQVKADTTTASEQAAQTQTNTAKKAAGTESTEQTEDNNANADAGKTAETPAATDNGSQETTTESTAASSSAQNQGQAATATSSTTTEAASSILSQADSETANSNTSQVVTATSSATTEAVSSAANQTGQKVSSSNNKSHDAKAHTTSAASGSISQVNDGQPITGLRHYSNNKLEYYGKDHVQYRNRYASQGNKWYYFGSNGDAVTGLRHYGNNKLEYYGKDHVQYRNRYASQGNKWYYFGSNGDAVTGLRHYGNNKLEYYGKDHVQYRNRYASQGNKWYYFGSNGDAVTGLRHYGNNKLEYYGKDHVQYRNRYASQGNKWYYFGSNGDAVTGLRHYGNNKLEYYGADHVQYRNRYYHEGNKFYYFGGNGDAKVTIRGAIEKGKFNIYDMRTNKLIKSLNAGTWENLPYSMDAKSINNIDGYLSYLGWYRPIGTSQNGKTWHKTRAVDWRPILMYAWTNKDVQAQFIKYFVNHGYKNANYGLTKASVANLNKGTNVTVLNKAAQNLRYVIEQSIAVNKGTGKLANDINGFAATVPELSASSELPYGQVIFVNNDNTSYADSKYRLMSRTINNQTGNDNSGSDNGYEFLTGIDIDNSNPVVQAENLNWEYFLLNYGKLMGYNPDGNFDGFRIDAADHIDADVLDQMGQLMDDMYHMKGNPQNANNHLSYNEGYRSGAARMLNKKGNPQLYMDYVGSTLGNVLGRANNRDTISNLITGSIVNRQNDVTENEATPNWSYVTNHDQRANLINGLISKDHPGAYKAEYANQAWQEFYADQKKTDKQYAQYNVPAQYAILLSNKDTVPQIYYGDLYNETAQYMQEKSIYYDAITTLMKARKQFVSGGQTMTKLSDNLIASVRYGKGVANANSEGTDSLSRTSGMAVIVGNNPQMAEQTISINMGRAHANEQYRNLLDTTDNGLTYNADGAENPETLTTDDNGILKVTVKGYSNPYVSGYLGVWVPVVSGNQDVTTNAATVSADSNKIFESNAALDSHMIYQDFSLYQPEPTSTENHAYNIIAQNAKLFNNLGITDFWMAPPYTPYSESRYKDGYSVTDRYNLGTNANPTKYGSGEELANAIAALHSAGLKVQVDIVMNQMIGLPGQEAVTVTRADNRGIQTYVNGKTYANQMYFAYTTGGGNGQETYGGKYLSELQSKYPDLFTTRAISTGVAPDPTTRITKWSAKYENGTSLQNIGIGLAVKLPNGDYAYLNGGNNDKFKTTLPEQMGSIDYYVQQELKNYVQQK

SEQ ID NO: 6 - protein, 1619 aa, Lactobacillus reuteri 121 (GtfB)
MELKKHFKLYKSGKQWVTAAVATIAFSAGVLTTSEVVHADTNTGDQQTEQVTQPSNSTTQDVKPVSTDASSDTKIVSDNKENNNQVGNTNVSGQNSSKDTKSVLTGTNSVTQNYDHNDNGNYGYIDSANLNNNQLQVSGWSATNQNINKDNHFIIAYDSTSQQELGRTKVETPVARPDVKAVHNVYNAENSGFNVNVSLNFDKMNNYRDAIKIISRYSGVPDGNSDYVDFVSQPIIFDENNYAHLDDFSVQNGKLHVSGWNATNKAIQNPNHFLILFDRTINREVARQKVTAGINRPDVEKAYPQVINANISGFDAAFDITTLNPNDEYQILSRYSNDDNGEGSYVTYWFKPQRIAPANQFNSGHLDSFNISKAGKVTVSGWQATNLSNIQSNRFIILFDNTANHQIASTKITNTARPDVEKVYPQVLNATNSGYDVTFDLTQDQIAQLLPNHSYSIVSRYSADANGNGNDKQHTDFWSTPITLNKTASYIDSISLNGNELNVRGWMASDASATQANPYLIVLNNGKEVTRQKLTLVARPDVAKVYPDVYSSLDSGFNTTIKLTVPQLNELTGNMQVLLRYSTAADGNPINNGGFTDQYSKNYATNGGSFDFVKVDNNQVAFSGWHVSDQATDKPYQWIIVLANGKEVGRQLISSTTNGFVSYNRPDVYNVNPAISNSSTSGFQGIMTLKDNIKNANVQLVHRFSDDGQNGEGNRVDYWSEVMPVTNTFQKGTDQLMRNLVAKPNKNQLKIYNGNTLVKTLGPGTWENMAFAQDSSAINNIDGYLSYTDWYRPYGTSQDGKTWYKTTAMDWRPLLMYIWPSKDVQAQFIKYFVNNGYENANYGLTKDTVANINKDTNTTVLANMAQNLRYVIEQSIAANKGTSKLANDINSFAATVPELSASSELSLQSMPNYRPDKSGTIDSDQVIFVNNNSKDPRKGNTSYADSNYRLMNRTINNQAGNNNSDNSPELLVGNDIDNSNPVVQAENLNWEYFLLNYGKLMGYNPDGNFDGFRVDAADNIDADVLDQMGQLMNDMYHTKGNPQNANDHLSYNEGYHSGAAQMLNEKGNPQLYMDSGEFYTLENVLGRANNRDNIGNLITNSIVNRQNDTTENEATPNWSFVTNHDQRKNLINRLIIKDHSNIPDIMGSAYKVEYANQAWQEFYADQEKTNKQYAQYNVPAQYAILLSNKDTVPQVYYGDLYNETAQYMQEKSIYYDAITTLMRARKQFVSGGQTMTKLNNNLLASVRYGKGVVDANSNGTDKLSRTSGMAVLVGNDSNMAQQSVAINMGRAHANQQYRNLIDTTENGLTYDADNSENPAILTTDSNGILKVTVKGYSNPYVSGYLGVWVPVISGDQDVTTNASDVVANKEKTFESNAALDSHMIYEDFSLFQPEPTSVENHAYNVIAKNASLFSDLGITDFWMAPAYTPFGRSRYNEGYSMTDRYNLGTTANPTKYGSGEELANTIAALHKAGLKVQEDIVMNQMIGFSGQEAVTVTRTNNRGMQIHVNGQTYANQIYFAYTTGGGNGQETYGGKYLAELQKNYPDLFTTKAISTGVAPDPTVRINKWSAKYQNGTSLQNIGIGLAVKLANGDYAYLNSGDNKAFNTLLPTAISLNFNN

SEQ ID NO: 7 - protein, 1620 aa, Lactobacillus reuteri ML1 (ML4)
MEIKKHFKLYKSGKQWVTASIATFAVSTGLVLGGGVVHAADNHPTTTSASVTNTVNNLKPQNDPEQQNNTQESNTVEFPKKDSQDNAVQPLKETAVMPNATNKDGAKASITNNAHTDNTIYGNIDPTTINDKELHVTGWNATNQAINKNESRYVIAYDDTTNSELGRTKITNQIARPDVEKVHKDIYNAQNSGFNVNISLDFNKMNNYRDAIKIISRYSGVPNGNSDYVDFVSQPIIFDENNYAYLDDFSVQNGRLHVSGRNATNKAIQRPNHFLILFDRTVNREVARQKVTAGINRSDVEKVYPQVVNANVSGFDATFDTINLNPNHEYQILSRYSNNGDGEGDYVTYWFNPQRIAPVNQFNNGHLDNFDISKAGKVTVSGWQATNLSNIQNNRYIILFDTTANCQIASMKVTGVDRPDVAKVYPQILNANKSGYNVTFDLTQAQIAQLFPNHSYSIVSRYSADPNGNGNDKQHTDFWSAPIVLNKTASYIDDISLNGDVLNVKGWMASDASATQANPYIIILNNGKEVTRQKLTLNDRPDVAKVYPDVYNSLASGFDTTIKLTNSQLNALNGNMQILLRYSAAADGNPINNGGFTDQYSKNYATNGGSFDFVKVDNNQVAFSGWHVSDQATDKPYQWIIVLVNGKEVGRQLISSTTNGLVSYNRPDVYNVNPAISNSSTSGFQGIMTLKDNIKNANVQLVHRFSDDGQNGEGNRVDYWSEVMPVTNTFQKGTDQLMRNLVAKPNKNQLKIYNGNTLVKTLGPGTWENMAFAQDSSAINNIDGYLSYTGWYRPYGTSQDGKTWYETTAMDWRPLLMYIWPSKDVQAQFIKYFVNNGYENANYGLTESSVASFSKDTNANLLDVTAQNLRYVIEQSIAANKGTSKLANDINSFAATVPELSASSELSLQSMPNYRPDESGTVDSDQVIFVNNNSKDPRKGNTGYADSNYRLMNRTINNQAGNNNSDNSPELLVGNDIDNSNPVVQAENLNWEYFLLNYGKLMGYNPDGNFDGFRVDAADNIDADVLDQMGQLMNDMYHTKGNPQNANDHLSYNEGYHSGAAQMLNEKGNPQLYMDSGEFYTLENVLGRANNRDSIGNLITNSVVNRQNDTTENEATPNWSFVTNHDQRKNLINRLIIKGHPNIPDIMGSAYKAEYANQAWQEFYADQKKTNKQYDQYNVPAQYAILLSNKDTVPQVYYGDLYNETAQYMQEKSIYYDTITTLMKARKQFVSGGQTMTKLNNNLLASVRYGKGVADSNSNGTDKLSRTSGIAVLVGNDSNMAQQTVAINMGRAHANQQYRNLIDTTENGLTYDGENSENPAILTTDSNGILKVTVKGYSNPYVSGYLGVWVPVISGDQDVTTSASDVVADKEKTFESNAALDSHMIYEDFSLFQPEPTNVENHAYNVIAKNANLFNDLGITDFWMAPAYTPFGMSRYNEGYSMTDRYNLGTTANPTKYGSGEELANTIAALHKVGLKVQEDIVMNQMIGFSGQEAVTVTRTNNRGMQIHVNGQTYANQIYFAYTTGGGNGQETYGGKYLAELQKNYPDLFTTKAISTEVVPDPTVRINKWSAKYENGTSLQNIGIGLAVKLANGDYAYLNSGDNKAFNTLLPTAISLNFNN

SEQ ID NO: 8 - protein, 1363 aa, Lactobacillus reuteri DSM 20016
MNLPTIPNTNVQTDNNWYLVDNGIAQSGVQQWAGSYYYFNPSTYLRVDNEYRQSQWGDWYMFGKDGRAVTGLYDYNGNTYYANPTTYLRETNKYISTSKGNMLLGNDGAALSGIQSVNGKYYYFDPVTHLQANKENYVQSQWGDWYLIGNDGQVLSGVQQWAGTYYYFDPTTYLRVDNDYRQSQWGLWYMFGHDGRIVTKVYPWAGTYYYFDPTTYLRVDNAYLQSQWGDWYLFGNDGRIQSGVQRWAGTYYYFDPTTYLRVDNDYVTSQWGSKYMFGPDGRIVTGLYKWSKNNQLYYFDPVTYLAVTNNYIKANNGNWYLFTADGTAASKVAPWAGSYYYFDPVTHLRVDNAYVQSQWGDWYMFGPDGRIVTGLKEWYGSYYYFDPTTYLKVTNKWIDNKYFGPDGRQAISSLENINNKFYCFDGNGQIIRNQFKKIDTHTYYFGSDGAALVGKQTIDGKNYHFASNGQLLGNLYGKIVDGKFNIYDSLSNKLIKTLDSGDWENMAYSQDSSSINNTDGYLSYSGWYRPYGTSQDGKTWYKTTASDWRPLLMYTWPSKDVEAKFIKYFVDNGYTNTDYGLTKDNVTNLSQDTDTQTLNKYARNLRFVIEKSIAANKSTGPLANDINKFMLTIPELSAKSELPVEYSNGYVPDVSGSIDNNQLIFINNNSDNQAKGNTSYADSNYRLMNRTINNQTNNDNSDQSPELLVGNDIDNSNPAVQAENFNWEYFLLNYGKLMKYNADGNFDGFRVDAADNIDADVLDQLGQLVNDMYHTKGNQENANNHLVYNEGYHSGAARMLNDKGNPELFMDAGYFYTLENVLGQAENKRDNVNNLITNSVVNRANDITENTATPNWSFVTNHDQRKNVINQIIIDNHPNIPDIMANSYKSTYAQKAWDEFYADQAKADKKYAQYNLPAQYALLLSNKDTVPQVYYGDLYKETDQYMKTKSMYYDAITTLMKARGEFVNGGQTMTKVNDNLITSVRYGKGVVDVSSNGTDPLSRTTGMAVIVGNNPSMSEQVVAINMGLAHANEQYRNLIDSTADGLTYNSNGSVNPSVLTTDSKGILRVTVKGYSNPYVSGYLSVWVPLINGTQNARTSAQEVRNVPGKVFTSNAALDSHMIYEDFSLFQPEPTTVNEHAYNVIKDNVALFNQLGITDFWMAPSYTPFNTSRYNEGYAMTDRYNLGTADNPTKYGNGEELSNAIAALHQAGLKVQEDLVMNQMIGFSTQEAVTVTRVDRDAKQLSVDGQTFADQIYFGYTRGGGQGQQDYGGKYLAELKQKYPDLFTTKAASTGVAPDPNTRITEWSAKYENGTSLQNVGIGLAVKMPNGYYAYLNDGNNKAFATTLPDAISSADYYANQENI

SEQ ID NO: 9 - protein, 1593 aa, Lactobacillus fermentum
MEFKKHFKLYKSGKQWCIAAVVTFTATLGLVAGNTTVNADTLTTGGSTPQAQVNQEKGITNTSQPASDQGKTSNTGDVRNTVPQPNNSDKTNQYQADTLTTGGSTPQAQVNQEKGITNTSQPASDQGKTSNTGDVRNTVPQPNNSGKTNQSQNGQDQKESAGNDNGSTGNNDQNKGQQTTDWQKNANNQWVYNGKTDQDLKGTQYVQLPTIPDTNVQGNTNWYFVKDGIAQSGVQQWAGTYYYFDPTTYLRVDNDYRQSQWGDWYLFGNDGRILSGVQQWAGTYYYFDPTTYLRVDDDYVTSQWGLKYMFGKDGRIATGLYKWDKNNQWYYFNPTTYLAVTNNYIQANDGHWYLFTADGTAASRVAKWAGTYYYFDPQTHLRVDDNYVQSQWGDWYMFGKDGRIATGLYKWDKNNQWYYFDPTTYLAVTNNYIQANDGHWYLFTADGTAASRVAKWAGTYYYFDPVTHLRVDNNYVQSQWGDWYLFGNDGRILSGVQQWAGTYYYFDPTTYLRVDDDYVTSQWGLKYMFGKDGRIATGLYKWDKNNQWYYFDPTTYLAVTNNYIQANDGHWYLFTADGTAASRVAKWAGTYYYFDPQTHLRVDDNYVQSQWGDWYMFGKDGRIATGLYKWDKNNQWYYFDPVTYLKVTNKWVDGNYYDEDGAQAISKLVTINNRLYYFDDQGKEISNQFRTIHGDKYYFGNDSAAVTGQQTIDGKVYKFSNYGYLLGNRYGKIENGKLNIYSLADHSLIKTVEAGPWENMAYSMDSNSINNIDGYISYTGWYRPYGTSQDGKTWYPTTVADWRPILMYVWPSKDVQVKFIQYFVNHGYENSNYGLTAGSVKDLSENTASINLNEVAQNLRYVIEQHIVAAKSTSQLANDINNFITTIPELSASSELPDESGSGQVIFVNNDNTSYADSKYRLMNRTVNNQTGNDNSDYCPEFVVGNDIDNSNPVVQAENLNWEYFLLNYGKLMGYNQDGNFDGFRIDAADDMDADVLDQIGQLMNDMYHMKGNPQNANNHLSYNEGYGPGAARMLNKKGNPQLFMDARECNTLENVLGRANNRDTISHLVTDSIVNRQNDVTENEATPNWSYVTNHDIRNNLINGLIIKDHPGMGSAYKAEYANQAWQEFYADQKKTDKQYAQYNVPAQYAILLSNKDTVPQIYYGDLYNETAQYMQEKSIYYDAITTLMKARKQFVSGGQTMTKLSDNLIASVRYGKGVANANSEGTDSLSRTSGMAVIVGNNPQMAEQTISINMGRAHANEQYRNLLDTTDNGLTYNADGAENPETLTTDDNGILKVTVKGYSNPYVSGYLGVWVPVASGNQDVTTNAATVSADSNKIFESNAALDSHMIYEDFSMYQPKPTSTENHAYNIIAQNAELFNNLGITDFWMAPAYTQAGTSRYNEGYSVADRYNLGTNANPTKYGSGEELANAIAALHSAGLKVQEDIVMNQMIGLPGQEAVTVTRADNRGMQTYVNGKTYANQMYFAYTTGGGNGQETYGGKYLSELQSKYPDLFTTRAISTGVAPDPTTHITKWSAKYENGTSLQNIGIGLAVKLANGDYAYLNDSNNKAFNTTLPETMSSTDYYANIEDN

SEQ ID NO: 10 - protein, 893 aa, Exiguobacterium sibiricum 255-15
MKNTKKVSAGLLATLVATSSFGVAPKQAAAYTSGEKLDNHVIFQSFSLYQPYDSNMYRTLAKKGDLLNSWGVTDVWMPPAYRSFDMARYMEGYAIADRYDLGEFPQGPGGTTATKYGKASHLEMMVDMLHDDNIKVQMDLVPNQMLGLNKREAVFVRRATSSGELFTNPYTGGQTTKTLATPYLAYTKGGGQGQEKYGYLKEWNKTFLNGTSLQGQGTGRVMTDKDGKPYRYFGPENEKNYLPEWLIEASKTQNLNVVDTYLAADGWYEVSPQNWKPMLSQYAKDPGYLAYMKENGFETKEALLASADNGTIAKLTEEYMKTQATYGYGTEERSYQNDNSGIDIEDQFLFVDETGFPLQAYNKTMTNNDEFLLGVDLANSNTEVIKEQKNWMKWMLETYKFDGFRIDAASHYDTAILKAEAQVAKEHFGKKEHLSYIESYKSEQKAYMKANNDEQLIMDSPLYFTMRTALGNEASKRPLSAIATGSTINRAGNGSTDVSANWSFVNNHDQEKNRVNQIMLDLYGIKTGIQYKAGEEPKSFEKMYDKDTEKQALGIYNAELASTKKKYSVDNVVSQYAFLLTNKDTVPTVYYGDLYQTDASYMSKQTPYYDEITNLLKVRKQYAYGAQKVAYHTTNTSKVAGSHLISSVRLGKDRNTGVATVIGKKSTLNTTIKVDMGKQHTNQVFVDASGVTQTKLVTDKNGILTVPVKGMRTAEVNGYLGVFVPQTTKAPTATIEKASVYQGKGINLKTKVLNTSSTVSSIRYQVADTSKATVDTTGRLVGKASGKTTVTATVTLKDGFVLTTTLPIETKVNEVKLKATQKTLKKGQTTTIGYASATDKIKSVSYASLNKKIATVNTKGQVKAVTKGTTSIRVTYTTVGNYKVVKTFKVIVK

SEQ ID NO: 11 - protein, 780 aa, Azotobacter chroococcum
MRASPSQFFAISLLSIAISGLLSGAAVAAPAPTALEQVPDGKGGVKWQEVTHDASAEEEQKGQDPKKFLGIQAITTEPDGSVKVEMGKPEVRQPASGDVFVSNEKLDEHVIFQAFALYQPNDNATYKALTENAPQLAQWGITDVWSPPPYRAASDSKYGEGYAIADRYDLGAYDKGPTKYGTADELKAAIGALHNNDIRIQVDVVPNQIIGLNERHVLPVTGVDMYGKPMNPFLDHYLYSTYSKGSAPGQAEHGVIKEWDYFHFHGTTTQYQGLFRVLSDANSTLYRYLGPNHPENYLPAFLAESDAAKYGKINTIDGYLLADTWFAVENAESENAVYAPLFLYYEEPRNGVVEQTFMDFARENGYTGSDEDIRATMLAELRMTPNPIGPLMDEYLAAQPGYSKKSEDDAKVTALRYDGPENDASHIGTNVLDFEFLVGNDLDTIREDVQQEQLNWQKYLLDFGFDGFRIDAASHINTDMLRDEVTQRLNHFAGEDVNEHLSYIESYVTQQVDFLQSNNYGQMAMDAGPFSGLMFSFGRDWAPLRYAFEASLIDRVNGGPALPNWSFVNNHDQEHNILVTVPLTEEEAGGYEPNSQPYELRQLEKYDADRNSVEKQWAPHNVPAMYAILLTTKDTVPTVFYGDMFVSSKPYMSTPTPYRDDIVNILKLRKQFAKGEQVIRYENSNTGSNGEDLVSNIRLGNDRKTGVAVVAGNNPALDTTITVDMGAQHRNQWFVDAMGYQPERLKTDKDGRLTVQVKGTQNVDVKGYLAAWVPDLQAQE

SEQ ID NO: 12 - protein, 708 aa, Paenibacillus beijingensis
MKVSLSLSLLAGTAIAGVAPANAAESNAKGFVSNAELDKHVIFQSFSLYQPYEKNMYNILGKNSAKLKDWGITDIWMPPAYRTFSGSYYGEGYAISDRYDLGEFPNGLNGERATKYGTSDELKRAIKQLHSKDLNVQVDLVPNQMMGFPKQEIVNVTAVDSYGNEIDPAFKDKLVPLYTKGGGPGQAKYGLIKEWSSKYFNGGGPMQMGSMRIMVDAEGKPYRYFGPDHQDNYLPEWLASSEAQKYGKINHIDNYLTVDSYFAVKGANTDNDQVWRSLLLYYVDPQAGSANESYLDFMRKNGFEGATDDEVREKIIAADSAAVTKLTDSYINAQPGYSAATDPKGLHRYNNGVNGNVNQNVLQYEFLVGTDIDNSNPTVQAEQLNWVKFLIDKYGFDGFRIDAASHYNTKILTDMRDEMSSRFGDDLNNHLSYIESYTDNQLGFENSTGNGQLVYDHGVFGALRDSLGKEHNWRPLSDIVTSSYVNRANPDAKPTPNWSFVMNHDQEHNGIKGIPLTEEEAGGTKKNTVDYEKKQFEKYYADMVNADKKYANYNVPSQYAYLLTNKDTVPTVYYGDMFKSTASYMSEKTQYFEPIVKLLQARQKYVSGDQKITYYNSNTSWSAGWDLLASVRFGTSRDTGVATVIGSNPNTQELISVDMGKLHANQTFEDVMGFNTQKLTTDENGVLTVPVKGVSNPLVHGYLGVWVP

SEQ ID NO: 13 - protein, 1772 aa, Lactobacillus reuteri 180 (Gtf180)
MEIKKHFKLYKSGKQWVTAAVATVAVSTALLYGGVAHADQQVQSSTTQEQTSTVNADTTKTVNLDTNTDQPAQTTDKNQVANDTTTNQSKTDSTSTTVKNPTFIPVSTLSSSDNEKQSQNYNKPDNGNYGNVDAAYFNNNQLHISGWHATNASQGTDSRQVIVRDITTKTELGRTNVTNNVLRPDVKNVHNVYNADNSGFDVNINIDFSKMKDYRDSIEIVSRYSGNGKSVDWWSQPITFDKNNYAYLDTFEVKNGELHATGWNATNKAINYNHHFVILFDRTNGKEVTRQEVRDGQSRPDVAKVYPQVVGANNSGFDVTFNIGDLDYTHQYQILSRYSNADNGEGDYVTYWFAPQSIAPANQSNQGYLDSFDISKNGEVTVTGWNATDLSELQTNHYVILFDQTAGQQVASAKVDLISRPDVAKAYPTVKTAETSGFKVTFKVSNLQPGHQYSVVSRFSADENGNGNDKRHTDYWYSPVTLNQTASNIDTITMTSNGLHITGWMASDNSINEATPYAIILNNGREVTRQKLTLIARPDVAAVYPSLYNSAVSGFDTTIKLTNAQYQALNGQLQVLLRFSKAVDGNPNGTNTVTDQFSKNYATTGGNFDYVKVNGNQIEFSGWHATNQSNDKNSQWIIVLVNGKEVKRQLVNDTKDGAAGFNRNDVYKVNPAIENSIMSGFQGIITLPVTVKDENVQLVHRFSNDAKTGEGNYVDFWSEVMSVKDSFQKGNGPLNQFGLQTINGQQYYIDPTTGQPRKNFLLQNGNDWIYFDKDTGAGTNALKLQFDKGTISADEQYRRGNEAYSYDDKSIENVNGYLTADTWYRPKQILKDGTTWTDSKETDMRPILMVWWPNTVTQAYYLNYMKQYGNLLPASLPSFSTDADSAELNHYSELVQQNIEKRISETGSTDWLRTLMHEFVTKNSMWNKDSENVDYGGLQLQGGFLKYVNSDLTKYANSDWRLMNRTATNIDGKNYGGAEFLLANDIDNSNPVVQAEELNWLYYLMNFGTITGNNPEANFDGIRVDAVDNVDVDLLSIARDYFNAAYNMEQSDASANKHINILEDWGWDDPAYVNKIGNPQLTMDDRLRNAIMDTLSGAPDKNQALNKLITQSLVNRANDNTENAVIPSYNFVRAHDSNAQDQIRQAIQAATGKPYGEFNLDDEKKGMEAYINDQNSTNKKWNLYNMPSAYTILLTNKDSVPRVYYGDLYQDGGQYMEHKTRYFDTITNLLKTRVKYVAGGQTMSVDKNGILTNVRFGKGAMNATDTGTDETRTEGIGVVISNNTNLKLNDGESVVLHMGAAHKNQKYRAVILTTEDGVKNYTNDTDAPVAYTDANGDLHFTNTNLDGQQYTAVRGYANPDVTGYLAVWVPAGAADDQDARTAPSDEAHTTKTAYRSNAALDSNVIYEGFSNFIYWPTTESERTNVRIAQNADLFKSWGITTFELAPQYNSSKDGTFLDSIIDNGYAFTDRYDLGMSTPNKYGSDEDLRNALQALHKAGLQAIADWVPDQIYNLPGKEAVTVTRSDDHGTTWEVSPIKNVVYITNTIGGGEYQKKYGGEFLDTLQKEYPQLFSQVYPVTQTTIDPSVKIKEWSAKYFNGTNILHRGAGYVLRSNDGKYYNLGTSTQQFLPSQLSVQDNEGYGFVKEGNNYHYYDENKQMVKDAFIQDSVGNWYYFDKNGNMVANQSPVEISSNGASGTYLFLNNGTSFRSGLVKTDAGTYYYDGDGRMVRNQTVSDGAMTYVLDENGKLVSESFDSSATEAHPLKPGDLNGQK

SEQ ID NO: 14 - protein, 1781 aa, Lactobacillus reuteri 121 (GtfA)
MEIKKHFKLYKSGKQWVTAAVATVAVSTALLYGGVAHADQQVQQASTTQDQTSTVNNDTDKTVALDTNTDQSAQTTDKKQVVSNTNQSKTDDTSTADKNSTSTPVSVLPSNNTEKQAKNYNEQDKGNYGNIDTAYFSNNQLHVSGWNATNASQGTNSRQIIVRDITTNNELGRTDVTNNVARPDVKNVHNVYNADNSGFDVNVNIDFSKMKDYRDSIEIVSRYSGNGKSVDWWSQPITFDKNNYAYLDTFEVKNGELHATGWNATNSAINYNHHFVILFDQTNGKEVARQEVREGQSRPDVAKVYPQVVGAANSGFNVTFNISDLDYTHQYQVLSRYSNSDNGEGDNVTYWFNPQSIAPANQSNQGYLDSFDISKNGEVTVTGWNATDLSELQNNHYVILFDQTAGKQVASAKADLISRPDVAKAYPTVKTATNSGFKVTFKVNNLQPGHQYSVVSRFSADENGNGNDKRHTDYWFSPVILNQTASNIDTITMTSNGLHIAGWMASDNSINETTPYAIILNNGKEVTRQKMSLTARPDVAAVYPSLYNSAVSGFDTTIKLTNDQYQALNGQLQVLLRFSKAADGNPSGDNTVTDQFSKNYATTGGNFDYVKVNGNQVEFSGWHATNQSNDKDSQWIIVLVNGKEVKRQLVNDTKEGAAGFNRNDVYKVNPAIENSSMSGFQGIITLPVTVKNENVQLVHRFSNDVKTGEGNYVDFWSELMPVKDSFQKGNGPLKQFGLQTINGQQYYIDPTTGQPRKNFLLQSGNNWIYFDSDTGVGTNALELQFAKGTVSSNEQYRNGNAAYSYDDKSIENVNGYLTADTWYRPKQILKDGTTWTDSKETDMRPILMVWWPNTLTQAYYLNYMKQHGNLLPSALPFFNADADPAELNHYSEIVQQNIEKRISETGNTDWLRTLMHDFVTNNPMWNKDSENVNFSGIQFQGGFLKYENSDLTPYANSDYRLLGRMPINIKDQTYRGQEFLLANDIDNSNPVVQAEQLNWLYYLLNFGTITANNDQANFDSVRVDAPDNIDADLMNIAQDYFNAAYGMDSDAVSNKHINILEDWNHADPEYFNKIGNPQLTMDDTIKNSLNHGLSDATNRWGLDAIVHQSLADRENNSTENVVIPNYSFVRAHDNNSQDQIQNAIRDVTGKDYHTFTFEDEQKGIDAYIQDQNSTVKKYNLYNIPASYAILLTNKDTIPRVYYGDLYTDGGQYMEHQTRYYDTLTNLLKSRVKYVAGGQSMQTMSVGGNNNILTSVRYGKGAMTATDTGTDETRTQGIGVVVSNTPNLKLGANDKVVLHMGAAHKNQQYRAAVLTTTDGVINYTSDQGAPVAMTDENGDLYLSSHNLVVNGKEEADTAVQGYANPDVSGYLAVWVPVGASDNQDARTAPSTEKNSGNSAYRTNAAFDSNVIFEAFSNFVYTPTKESERANVRIAQNADFFASLGFTSFEMAPQYNSSKDRTFLDSTIDNGYAFTDRYDLGMSEPNKYGTDEDLRNAIQALHKAGLQVMADWVPDQIYNLPGKEVATVTRVDDRGNVWKDAIINNNLYVVNTIGGGEYQKKYGGAFLDKLQKLYPEIFTKKQVSTGVAIDPSQKITEWSAKYFNGTNILHRGSGYVLKADGGQYYNLGTTTKQFLPIQLTGEKKQGNEGFVKGNDGNYYFYDLAGNMVKNTFIEDSVGNWYFFDQDGKMVENKHFVDVDSYGEKGTYFFLKNGVSFRGGLVQTDNGTYYFDNYGKMVRNQTINAGAMIYTLDENGKLIKASYNSDAEYPTSTDVGKMLDQNKL

SEQ ID NO: 15 - protein, 1455 aa, streptococcus mutans SI (GtfSI)
MEKKVRFKLRKVKKRWVTVSVASAVVTLTSLSGSLVKADSTDDRQQAVTESQASLVTTSEAAKETLTATDTSTATSATSQPTATVTDNVSTTNQSTNTTANTANFDVKPTTTSEQSKTDNSDKIIATSKAVNRLTATGKFVPANNNTAHSRTVTDKIVPIKPKIGKLKQPSSLSQDDIAALGNVKNIRKVNGKYYYYKEDGTLQKNYALNINGKTFFFDETGALSNNTLPSKKGNITNNDNTNSFAQYNQVYSTDAANFEHVDHYLTAESWYRPKYILKDGKTWTQSTEKDFRPLLMTWWPDQETQRQYVNYMNAQLGIHQTYNTATSPLQLNLAAQTIQTKIEEKITAEKNTNWLRQTISAFVKTQSAWNSDSEKPFDDHLQKGALLYSNNSKLTSQANSNYRILNRTPTNQTGKKDPRYTADRTIGGYEFLLANDVDNSNPVVQAEQLNWLHFLMNFGNIYANDPDANFDSIRVDAVDNVDADLLQIAGDYLKAAKGIHKNDKAANDHLSILEAWSYNDTPYLHDDGDNMINMDNRLRLSLLYSLAKPLNQRSGMNPLITNSLVNRTDDNAETAAVPSYSFIRAHDSEVQDLIRNIIRAEINPNVVGYSFTMEEIKKAFEIYNKDLLATEKKYTHYNTALSYALLLTNKSSVPRVYYGDMFTDDGQYMAHKTINYEAIETLLKARIKYVSGGQAMRNQQVGNSEIITSVRYGKGALKATDTGDRTTRTSGVAVIEGNNPSLRLKASDRVVVNMGAAHKNQAYRPLLLTTDNGIKAYHSDQEAAGLVRYTNDRGELIFTAADIKGYANPQVSGYLGVWVPVGAAADQDVRVAASTAPSTDGKSVHQNAALDSRVMFEGFSNFQAFATKKEEYTNVVIAKNVDKFAEWGVTDFEMAPQYVSSTDGSFLDSVIQNGYAFTDRYDLGISKPNKYGTADDLVKAIKALHSKGIKVMADWVPDQMYALPEKEVVTATRVDKYGTPVAGSQIKNTLYVVDGKSSGKDQQAKYGGAFLEELQAKYPELFARKQISTGVPMDPSVKIKQWSAKYFNGTNILGRGAGYVLKDQATNTYFSLVSDNTFLPKSLVNPNHGTSSSVTGLVFDGKGYVYYSTSGNQAKNAFISLGNNWYYFDNNGYMVTGAQSINGANYYFLSNGIQLRNAIYDNGNKVLSYYGNDGRRYENGYYLFGQQWRYFQNGIMAVGLTRIHGAVQYFDASGFQAKGQFITTADGKLRYFDRDSGNQISNRFVRNSKGEWFLFDHNGVAVTGTVTFNGQRLYFKPNGVQAKGEFIRDADGHLRYYDPNSGNEVRNRFVRNSKGEWFLFDHNGIAVTGTRVVNGQRLYFKSNGVQAKGELITERKGRIKYYDPNSGNEVRNRYVRTSSGNWYYFGNDGYALIGWHVVEGRRVYFDENGVYRYASHDQRNHWDYDYRRDFGRGSSSAVRFRHSRNGFFDNFFRF

SEQ ID NO: 16 - protein, 2057 aa, Leuconostoc mesenteroides
MKQQETVTRKKLYKSGKVWVAAATAFAVLGVSTVTTVHADTNSNVAVKQINNTGTNDSGEKKVPVPSTNNDSLKQGTDGFWYDSDGNRVDQKTNQILLTAEQLKKNNEKNLSVISDDTSKKDDENISKQTKIANQQTVDTAKGLTTSNLSDPITGGHYENHNGYFVYIDASGKQVTGLQNIDGNLQYFDDNGYQVKGSFRDVNGKHIYFDSVTGKASSNVDIVNGKAQGYDAQGNQLKKSYVADSSGQTYYFDGNGQPLIGLQTIDGNLQYFNQQGVQIKGGFQDVNNKRIYFAPNTGNAVANTEIINGKLQGRDANGNQVKNAFSKDVAGNTFYFDANGVMLTGLQTISGKTYYLDEQGHLRKNYAGTFNNQFMYFDADTGAGKTAIEYQFDQGLVSQSNENTPHNAAKSYDKSSFENVDGYLTADTWYRPTDILKNGDTWTASTETDMRPLLMTWWPDKQTQANYLNFMSSKGLGITTTYTAATSQKTLNDAAFVIQTAIEQQISLKKSTEWLRDAIDSFVKTQANWNKQTEDEAFDGLQWLQGGFLAYQDDSHRTPNTDSGNNRKLGRQPINIDGSKDTTDGKGSEFLLANDIDNSNPIVQAEQLNWLHYLMNFGSITGNNDNANFDGIRVDAVDNVDADLLKIAGDYFKALYGTDKSDANANKHLSILEDWNGKDPQYVNQQGNAQLTMDYTVTSQFGNSLTHGANNRSNMWYFLDTGYYLNGDLNKKIVDKNRPNSGTLVNRIANSGDTKVIPNYSFVRAHDYDAQDPIRKAMIDHGIIKNMQDTFTFDQLAQGMEFYYKDQENPSGFKKYNDYNLPSAYAMLLTNKDTVPRVYYGDMYLEGGQYMEKGTIYNPVISALLKARIKYVSGGQTMATDSSGKDLKDGETDLLTSVRFGKGIMTSDQTTTQDNSQDYKNQGIGVIVGNNPDLKLNNDKTITLHMGKAHKNQLYRALVLSNDSGIDVYDSDDKAPTLRTNDNGDLIFHKTNTFVKQDGTIINYEMKGSLNALISGYLGVWVPVGASDSQDARTVATESSSSNDGSVFHSNAALDSNVIYEGFSNFQAMPTSPEQSTNVVIATKANLFKELGITSFELAPQYRSSGDTNYGGMSFLDSFLNNGYAFTDRYDLGFNKADGNPNPTKYGTDQDLRNAIEALHKNGMQAIADWVPDQIYALPGKEVVTATRVDERGNQLKDTDFVNLLYVANTKSSGVDYQAKYGGEFLDKLREEYPSLFKQNQVSTGQPIDASTKIKQWSAKYMNGTNILHRGAYYVLKDWATNQYFNIAKTNEVFLPLQLQNKDAQTGFISDASGVKYYSISGYQAKDTFIEDGNGNWYYFDKDGYMVRSQQGENPIRTVETSVNTRNGNYYFMPNGVELRKGFGTDNSGNVYYFDDQGKMVRDKYINDDANNFYHLNVDGTMSRGLFKFDSDTLQYFASNGVQIKDSYAKDSKGNKYYFDSATGNNDTGKAQTWDGNGYYITIDSDANNTIGVNTDYTAYITSSLREDGLFANAPYGVVTKDQNGNDLKWQYINHTKQYEGQQVQVTRQYTDSKGVSWNLITFAGGDLQGQRLWVDSRALTMTPFKTMNQISFISYANRNDGLFLNAPYQVKGYQLAGMSNQYKGQQVTIAGVANVSGKDWSLISFNGTQYWIDSQALNTNFTHDMNQKVFVNTTSNLDGLFLNAPYRQPGYKLAGLAKNYNNQTVTVSQQYFDDQGTVWSQVVLGGQTVWVDNHALAQMQVSDTDQQLYVNSNGRNDGLFLNAPYRGQGSQLIGMTADYNGQHVQVTKQGQDAYGAQWRLITLNNQQVWVDSRALSTTIMQAMNDNMYVNSSQRTDGLWLNAPYTMSGAKWAGDTRSANGRYVHISKAYSNEVGNTYYLTNLNGQSTWIDKRAFTVTFDQVVALNATIVARQRPDGMFKTAPYGEAGAQFVDYVTNYNQQTVPVTKQHSDAQGNQWYLATVNGTQYWIDQRSFSPVVTKVVDYQAKIVPRTTRDGVFSGAPYGEVNAKLVNMATAYQNQVVHATGEYTNASGITWSQFALSGQEDKLWIDKRALQA

SEQ ID NO: 17 - protein, 2835 aa, Leuconostoc citreum
MRDMRVICDRKKLYKSGKVLVTAGIFALMMFGVTTASVSANTIAVDTNHSRTSAQINKSAVDKVNDDKTTLGAAKVVAVATTPATPVADKTVSAPAADKAVDTTSSTTPATDKAVDTTPTTPAADKAVDTTPTTPAADKAVDTTPTTPAANKAVDTTPATAATDKAVATPATPAADKLANTTPATDKAVATTPATPVANKAADTSSIHDQPLDTNVPTDKSANLVSTTQKSTDNQQVKSTETSHLQEINGKTYFLDDNGQVKKNFTAIIDGKVLYFDKTSGELTANAPQVTKGLVNIDNAHNAAHDLTADNFTNVDGYLTANSWYRPKDILKNGTTWTPTTAEDFRPLLMSWWPDKNTQVAYLQYMQSVGMLPDDVKVSNDDNMSTLTDAAMTVQKNIESRIGVSGKTDWLKQDMNKLIDSQANWNIDSESKGNDHLQGGALLYVNDDKTPNANSDYRLLNRTPTNQTGQITDPSKQGGYEMLLANDVDNSNPVVQAEQLNWLHYMMNIGTIAQNDPTANFDGYRVDAVDNVDADLLQIAGDYFKAAYGTGKTEANANNHISILEDWDNNDSAYIKAHGNNQLTMDFPAHLALKYALNMPLAAQSGLEPLINTSLVKRGKDATENEAQPNYAFIRAHDSEVQTVIAQIIKDKINTKSDGLTVTPDEIKQAFTIYNADELKADKEYTAYNIPASYAVLLTNKDTVPRVYYGDLFSDDGQYMSQKSPYYDAITSLLKSRIKYVAGGQSMNMTYLHECFDPAKNETKPQGVLTSVRYGKGAMTADDLGNSDTRQQGIGLVINNKPFLNLNDDEQIVLNMGAAHKNQAYRPLMLTTKSGLQIYDKDAGAPVVYTNDAGQLIFKSDMVYGVSNPQVSGYFAAWVPVGASDSQDARTQSSQSETKDGDVYHSNAALDSNVIYEGFSNFQAMPEKNDDFTNVKIAQNAKLFKDLGITSFELAPQYRSSTDNSFLDSVIQNGYAFTDRYDVGYNTPTKYGTVDQLLDSLRALHAQGIQAINDWVPDQIYNLPGEQIVTAVRTNGSGKYDYDSVINNTLYDSRTVGGGEYQEKFGGLFLDQLKKDYPSLFETKQISTNQPMNPDVKIKEWSAKYFNGSNIQGRGAWYVLKDWATNQYFNVSSDNGFLPKQLLGEKTSTGFITENGKTSFYSTSGYQAKDTFIQDGTNWYYFDNAGYMLTGKQNIHDKNYYFLPNGVELQDAYLFDGNQEFYYNKAGEQVMNQYYQDSQNQWHYFFENGRMAIGLTEVPNADGTHVTQYFDANGVQIKGTAIKDQNNQLRYFDEATGNMVVNSWGQLADKSWLYLNAQGVAVTGNQKIDGEEYYFNADGKQVKGNAIIDNNGDQRYYDGDKGVMVVNSWGELPDGSWLYLNDKGIAVTGRQVINNQVNFFGNDGKQIKDAFKLLSDGSWVYLDDKGLITTGAKVINGLNMFFDKDGHQIKGDASTDANGKRHYYDKNDGHLVTNSWGELPDGSWLYLEEQGDAVTGQRVIDGKTRYFDEDGKQIKNSLKTLANGDKIYLDGDGVAATGLQHVGDKIMYFDEDGKQVVGKFVSAKDGSWYYLNQDGVAAVGPSSINGQSLYFDQDGKQVKYNEVRNSDGTTNYYTGLTGEKLTQDFGELPDGSWIYLDAQGHTVTGAQIINGQNLYFKADGQQVKGHAYTDQLGHMRFYDPDSGDMLSNRFEQITPGVWAYFGADGVAITGQHDINGQKLFFDETGYQVKGSQRTIDGTLYSFDSQTGNQKRVQTTLLPQAGHYITKNGNDWQYDTNGELAKGLRQDSNGKLRYFDLTTGIQAKGQFVTIGQETYYFSKDHGDAQLLPMVTEGHYGTITLKQGQDTKTAWVYRDQNNTILKGLQNINGTLQFFDPYTGEQLKGGVAKYDDKLFYFESGKGNLVSTVAGDYQDGHYISQDGQTRYADKQNQLVKGLVTVNGALQYFDNATGNQIKNQQVIVDGKTYYFDDKGNGEYLFTNTLDMSTNAFSTKNVAFNHDSSSFDHTVDGFLTADTWYRPKSILANGTTWRDSTDKDMRPLITVWWPNKNVQVNYLNFMKANGLLTTAAQYTLHSDQYDLNQAAQDVQVAIERRIASEHGTDWLQKLLFESQNNNPSFVKQQFIWNKDSEYHGGGDAWFQGGYLKYGNNPLTPTTNSDYRQPGNAFDFLLANDVDNSNPVVQAENLNWLHYLMNFGTITAGQDDANFDSIRIDAVDFIHNDTIQRTYDYLRDAYQVQQSEAKANQHISLVEAGLDAGTSTIHNDALIESNLREAATLSLTNEPGKNKPLTNMLQDVDGGTLITDHTQNSTENQATPNYSIIHAHDKGVQEKVGAAITDATGADWTNFTDEQLKAGLELFYKDQRATNKKYNSYNIPSIYALMLTNKDTVPRMYYGDMYQDDGQYMANKSIYYDALVSLMTARKSYVSGGQTMSVDNHGLLKSVRFGKDAMTANDLGTSATRTEGLGVIIGNDPKLQLNDSDKVTLDMGAAHKNQKYRAVILTTRDGLATFNSDQAPTAWTNDQGTLTFSNQEINGQDNTQIRGVANPQVSGYLAVWVPVGASDNQDARTAATTTENHDGKVLHSNAALDSNLIYEGFSNFQPKATTHDELTNVVIAKNADVFNNWGITSFEMAPQYRSSGDHTFLDSTIDNGYAFTDRYDLGFNTPTKYGTDGDLRATIQALHHANMQVMADVVDNQVYNLPGKEVVSATRAGVYGNDDATGFGTQLYVTNSVGGGQYQEKYAGQYLEALKAKYPDLFEGKAYDYWYKNYANDGSNPYYTLSHGDRESIPADVAIKQWSAKYMNGTNVLGNGMGYVLKDWHNGQYFKLDGDKSTLPQI

SEQ ID NO: 18 - protein, 1888 aa, Leuconostoc citreum
MEMKETITRKKLYKSGKSWVAAATAFAVMGVSAVTTVSADTQTPVGTTQSQQDLTGQTGQDKPTTKEVIDKKEPVPQVSAQNVGDLSADAKTPKADDKQDTQPTNAQLPDQGNKQTNSNSDKGVKESTTAPVKTTDVPSKSVAPETNTSINGGQYVEKDGQFVYIDQSGKQVSGLQNIEGHTQYFDPKTGYQTKGELKNIDDNAYYFDKNSGNGRTFTKISNGSYSEKDGMWQYVDSHDKQPVKGLYDVEGNLQYFDLSTGNQAKHQIRSVDGVTYYFDADSGNATAFKAVTNGRYAEQTTKDKDGNETSYWAYLDNQGNAIKGLNDVNGEIQYFDEHTGEQLKGHTATVDGTTYYFEGNKGNLVSVVNTAPTGQYKINGDNVYYLDNNNEAIKGLYGINGNLNYFDLATGIQLKGQAKNIDGIGYYFDQNNGNGEYRYSLTGPVVKDVYSQHNAVNNLSANNFKNLVDGFLTAETWYRPAQILSHGTDWVASTDKDFRPLITVWWPNKDIQVNYLKLMQQIGILDNSVVFDTNNDQLVLNKGAESAQIGIEKKVSETGNTDWLNELLFAPNGNQPSFIKQQYLWNVDSEYPGGWFQGGYLAYQNSDLTPYANTNPDYRTHNGLEFLLANDVDNSNPVVQAEQLNWLYYLMNFGQITANDSNANFDSMRIDAISFVDPQIAKKAYDLLDKMYGLTDNEAVANQHISIVEAPKGETPITVEKQSALVESNWRDRMKQSLSKNATLDKLDPDPAINSLEKLVADDLVNRSQSSDKDSSTIPNYSIVHAHDKDIQDTVIHIMKIVNNNPNISMSDFTMQQLQNGLKAFYEDQHQSVKKYNQYNIPSAYALLLTNKDTVPRVFYGDMYQDYGDDLDGGQYMATKSIYYNAIEQMMKARLKYVAGGQIMAVTKIKNDGINKDGTNKSGEVLTSVRFGKDIMDAQGQGTAESRNQGIGVIVSNSSGLELKNSDSITLHMGIAHKNQAYRALMLTNDKGIVNYDQDNNAPIAWTNDHGDLIFTNQMINGQSDTAVKGYLNPEVAGYLAVWVPVGANDNQDARTVTTNQKNTDGKVLHTNAALDSKLMYEGFSNFQKMPTRGNQYANVVITKNIDLFKSWGITDFELAPQYRSSDGKDITDRFLDSIVQNGYGLSDRYDLGFKTPTKYGTDQDLRKAIERLHQAGMSVMADFVANQIYGLHADKEVVSAQHVNINGDTKLVVDPRYGTQMTVVNSVGGGDYQAKYGGEYLDTISKLYPGLLLDSNGQKIDLSTKIKEWSAKYLNGSNIPQVGMGYVLKDWNNGQYFHILDKEGQYSLPTQLVSNDPETQIGESVNYKYFIGNSDATYNMYHNLPNTVSLINSQEGQIKTQQSGVTSDYEGQQVQVTRQYTDSKGVSWNLITFAGGDLQGQKLWVDSRALTMTPFKTMNQISFISYANRNDGLFLNAPYQVKGYQLAGMSNQYKGQQVTIAGVANVSGKDWSLISFNGTQYWIDSQALNTNFTHDMNQKVFVNTTSNLDGLFLNAPYRQPGYKLAGLAKNYNNQTVTVSQQYFDDQGTVWSQVVLGGQTVWVDNHALAQMQVSDTSQQLYVNSNGRNDGLFLNAPYRGQGSQLIGMTADYNGQHVQVTKQGQDAYGAQWRLITLNNQQVWVDSRALSTTIVQAMNDDMYVNSNQRTDGLWLNAPYTMSGAKWAGDTRLANGRYVHISKAYSNEVGNTYYLTNLNGQSTWIDKRAFTATFDQVVALNATIVARQRPDGMFKTAPYGEAGAQFVDYVTNYNQQTVPVTKQHSDAQGNQWYLATVNGTQYWIDQRSFSPVVTKAVDYQAKIVPRTTRDGVFSGAPYGEVNAKLVNMATAYQNQVVHATGEYTNASGITWSQFALSGQEDKLWIDKRALQA

SEQ ID NO: 19 - protein, 1244 aa, Lactobacillus reuteri
  CNCM I-2451
IPDTNVQGNTNWYFVKDGIAQSGVQQWAGSYYYFDPVTYLRVDNRYVQSQWGLKYMFGKDGRIATGLYKWDKNNQWYYFNPITYLAVTNDYIQANDGNWYLFTADGTAASRVAQWAGTYYYFDPVTHLRVDNNYVQSQWGDWYLFGNDGRILSGVQQWAGTYYYFDPTTYLRVDDDYVTSQWGLKYMFGKDGRIATGLYKWDKNNQWYYFDPTTYLAVTNNYIQANDGHWYLFTADGTAASRVAKWAGTYYYFDPVTHLRVDNNYVQSQWGDWYMFGNDGRIITGRTLWYGNYYYFDPVTYLKVTNKWVDGNYYDEDGAQAISKLVTINNRLYYFDDQGKEISNQFRTIYGNTYYFGNDSAAVTGQQTIDGKVYNFSKYGHLLGNRYGKIENGKLNIYSLADNSLIKTVEAGPWENMAYSMDSNSINNIDGYISYTGWYRPYGTSQDGKTWYPTTVADWRPILMYVWPSKDVQAKFIQYFVNHGYENSNYGLTTGSVKDLSENTASIKLNEVAQNLRYVIEQHIVAAKSTSQLANDINNFITTIPELSASSELPYGQVIFVNNDNTSYADSKYRLMSRTINNQTGNDNDNSDNGYEFLTGIDIDNSNPVVQAENLNWEYFLLNYGKLMGYNPDGNFDGFRIDAADHIDADVLDQTGQLMDDMYHMKGNPQNANNHLSYNEGYRSSAARMLNKKGNPQLYMDYVGSTLGNVLGRANNRDTISNLVTGSIVNRQNDVTENEATPNWSYVTNHDSRANLINGLISKDHPGAYKAEYANQAWQEFYADQKKTDKQYAQYNVPAQYAILLSNKDTVPQIYYGDLYNETAQYMQEKSIYYDAITTLMKARKQFVSGGQTMTKLSDNLIASVRYGKGVTNANSEGTDSLSRTSGMAVIVGNNPQMAEQTISINMGRAHANEQYRNLLDTTDNGLTYNADGAENPETLTTDDNGILKVTVKGYSNPYVSGYLGVWVPVVSGNQDVTTNAATVSADSNKIFESNAALDSHMIYQDFSLYQPEPTSTENHAYNTIAQNAELFNNLGITDFWMAPPYTQYSESRYNDGYSVTDRYNLGTNANPTKYGSGEELANAIAALHSAGLKVQVDIVMNQMIGLPGQEAVTVTRADNRGIQTYVNGKTYANQMYFAYTTGGGNGQETYGGKYLSELQSKYPDLFTTRAISTGVAPDPTTRITKWSAKYENGTSLQNIGIGLAVKLPNGEYAYLRSSDNKAFNTTLPETMSSADYYANIEDD